European Patent Application EP 4 530 349 A1, published April 2, 2025. Title: IMMOBILIZED ENZYME AND USE THEREOF AND METHOD THEREFOR FOR PREPARING ETHYLHEXYLGLYCERIN. Applicant: NANJING ASCEND MEGABIO TECHNOLOGY CO., LTD. The sequence listing filed with the application follows.

SEQUENCE LISTING (10 sequences)

SEQ ID NO: 1 - DNA, 1131 bp, Novosphingobium aromaticivorans
  source 1..1131: mol_type = genomic DNA; note = epoxide hydrolase (NaEH) gene from Novosphingobium aromaticivorans
atggatgttgcgcctttcgttgtcgacatacctcgcggcgagatcgaggacctgcatcgtcgcatcgacatgacacgctggcccgagaaagagacggtcgacgactggtcgcagggcacgccgcttggcgcgttgcaggatttcgtgagctactggcgcggcggctatgactggtacgcgtgccagaggatgctgaacgactggggcatgttcgagaccgagatcgacggagtggcgatccgcttcctccacgtgcgctctgcgcaagcagatgcgcggcccttgctgctgacccacggctggccgggatcgattctcgagttccgccgctgcatcgcgccgctgacccgcccagaggagcatggtggtactgccgccgacgcgttccatctcgtgatcccttgcctgccgggatacggcttttccggaaagcccacgcgcaagggctggagcgtgcagaagatcgcgcaggcctggggcgaactgatgaagcggctgggctacgaaagctggcttgcacagggcggggactggggttccgccgttaccactgccatcggggcgctgaaggtggagggctgcgcgggcatccatctcaacatgccgatcgcccggcccctgccggaggacctggccgctccgacgccggaggagctaagggcgctgaccgcgctacagcactatcaggattgggattcggggtattccaaggagcaggcgacccggccccagacggtaggttacgggctggtcgattcgccggtcgggctggctggctggatctacgagaagatgtgggcctggaccgacaacgagggcgcgcccgaggacgcgctgagccgcgacgacatgctcgacaacatcatgctgtactggctgacggcggcaggggcatcgtcggcccggctttattgggagagttttgcgagcttcgggccatcgcagatcgacattccggccgcggccagcgcctttccgaaggagataattcccgcgccgcgcaagtggttcgagcgcaactgttcgaagctggtctactggggcgagctggaaaagggcggccactttgccgcgtgggagcagcccgaagccttcgtgaaggaacttcgggccgcgttttccctgatgtgc

SEQ ID NO: 2 - DNA, 135 bp, Lactococcus lactis
  source 1..135: mol_type = genomic DNA; note = chitin-binding protein (LlChBD) gene from Lactococcus lactis
actacttataccgtcaaatctggtgatactctttggggaatctcacaaagatatggaattagtgtcgctcaaattcaaagtgcgaataatcttaaaagtaccattatctacattggtcaaaaacttgtactgaca

SEQ ID NO: 3 - DNA, 60 bp, synthetic construct
  source 1..60: mol_type = other DNA; note = DNA sequence of a synthetic linker peptide
ggaggtggtggatcaggaggtggtggatcaggaggtggtggatcagaagctgcagctaag

SEQ ID NO: 4 - DNA, 1329 bp, synthetic construct
  source 1..1329: mol_type = other DNA; note = DNA sequence of the fusion protein of the present disclosure
atggatgttgcgcctttcgttgtcgacatacctcgcggcgagatcgaggacctgcatcgtcgcatcgacatgacacgctggcccgagaaagagacggtcgacgactggtcgcagggcacgccgcttggcgcgttgcaggatttcgtgagctactggcgcggcggctatgactggtacgcgtgccagaggatgctgaacgactggggcatgttcgagaccgagatcgacggagtggcgatccgcttcctccacgtgcgctctgcgcaagcagatgcgcggcccttgctgctgacccacggctggccgggatcgattctcgagttccgccgctgcatcgcgccgctgacccgcccagaggagcatggtggtactgccgccgacgcgttccatctcgtgatcccttgcctgccgggatacggcttttccggaaagcccacgcgcaagggctggagcgtgcagaagatcgcgcaggcctggggcgaactgatgaagcggctgggctacgaaagctggcttgcacagggcggggactggggttccgccgttaccactgccatcggggcgctgaaggtggagggctgcgcgggcatccatctcaacatgccgatcgcccggcccctgccggaggacctggccgctccgacgccggaggagctaagggcgctgaccgcgctacagcactatcaggattgggattcggggtattccaaggagcaggcgacccggccccagacggtaggttacgggctggtcgattcgccggtcgggctggctggctggatctacgagaagatgtgggcctggaccgacaacgagggcgcgcccgaggacgcgctgagccgcgacgacatgctcgacaacatcatgctgtactggctgacggcggcaggggcatcgtcggcccggctttattgggagagttttgcgagcttcgggccatcgcagatcgacattccggccgcggccagcgcctttccgaaggagataattcccgcgccgcgcaagtggttcgagcgcaactgttcgaagctggtctactggggcgagctggaaaagggcggccactttgccgcgtgggagcagcccgaagccttcgtgaaggaacttcgggccgcgttttccctgatgtgcggaggtggtggatcaggaggtggtggatcaggaggtggtggatcagaagctgcagctaagactacttataccgtcaaatctggtgatactctttggggaatctcacaaagatatggaattagtgtcgctcaaattcaaagtgcgaataatcttaaaagtaccattatctacattggtcaaaaacttgtactgacataa

SEQ ID NO: 5 - DNA, 42 bp, synthetic construct
  source 1..42: mol_type = other DNA; note = NaEH forward primer (EHG-F)
gctaacaggaggaattaaccatggatgttgcgcctttcgttg

SEQ ID NO: 6 - DNA, 60 bp, synthetic construct
  source 1..60: mol_type = other DNA; note = NaEH reverse primer (EHG-R)
ccaccacctcctgatccaccacctcctgatccaccacctccgcacatcagggaaaacgcg

SEQ ID NO: 7 - DNA, 60 bp, synthetic construct
  source 1..60: mol_type = other DNA; note = LlChBD forward primer (LL-F)
ggtggatcaggaggtggtggatcagaagctgcagctaagactacttataccgtcaaatct

SEQ ID NO: 8 - DNA, 53 bp, synthetic construct
  source 1..53: mol_type = other DNA; note = LlChBD reverse primer (LL-R)
gctgcagaccgagctcaccgaattcttatgtcagtacaagtttttgaccaatg

SEQ ID NO: 9 - DNA, 20 bp, synthetic construct
  source 1..20: mol_type = other DNA; note = forward primer for verification (pBAD-F)
cggcgtcacactttgctatg

SEQ ID NO: 10 - DNA, 21 bp, synthetic construct
  source 1..21: mol_type = other DNA; note = reverse primer for verification (pBAD-R)
cgtttcacttctgagttcggc